European Patent Application EP 4 241 841 A1, published September 13, 2023. Title: 制备聚乙二醇修饰的尿酸氧化酶的方法. Applicant: 杭州远大生物制药有限公司. The sequence listing filed with the application follows.

SEQUENCE LISTING (7 sequences)

SEQ ID NO: 1 - protein, 298 aa, Artificial
  1
TYKKNDEVEFVRTGYGKDMIKVLHIQRDGKYHSIKEVATTVQLTLSSKKDYLHGDNSDVIPTDTIKNTVNVLAKFKGIKSIETFAVTICEHFLSSFKHVIRAQVYVEEVPWKRFEKNGVKHVHAFIYTPTGTHFCEVEQIRNGPPVIHSGIKDLKVLKTTQSGFEGFIKDQFTTLPEVKDRCFATQVYCKWRYHQGRDVDFEATWDTVRSIVLQKFAGPYDKGEYSPSVQKTLYDIQVLTLGQVPEIEDMEISLPNIHYLNIDMSKMGLINKEEVLLPLDNPYGKITGTVKRKLSSRL

SEQ ID NO: 2 - protein, 304 aa, Artificial
  2
MAHYRNDYKKNDEVEFVRTGYGKDMIKVLHIQRDGKYHSIKEVATSVQLTLSSKKDYLHGDNSDVIPTDTIKNTVNVLAKFKGIKSIETFAVTICEHFLSSFKHVIRAQVYVEEVPWKRFEKNGVKHVHAFIYTPTGTHFCEVEQIRNGPPVIHSGIKDLKVLKTTQSGFEGFIKDQFTTLPEVKDRCFATQVYCKWRYHQGRDVDFEATWDTVRSIVLQKFAGPYDKGEYSPSVQKTLYDIQVLTLGQVPEIEDMEISLPNIHYLNIDMSKMGLINKEEVLLPLDNPYGRITGTVKRKLTSRL

SEQ ID NO: 3 - protein, 297 aa, Artificial
  3
MYKNDEVEFVRTGYGKDMVKVLHIQRDGKYHSIKEVATSVQLTLSSKKDYVYGDNSDIIPTDTIKNTVHVLAKFKGIKSIETFAMNICEHFLSSFNHVIRAQVYVEEVPWKRFEKNGVKHVHAFIHNPTGTHFCEVEQMRSGPPVIHSGIKDLKVLKTTQSGFEGFIKDQFTTLPEVKDRCFATKVYCKWRYHQGRDVDFEATWDTVRDIVLEKFAGPYDKGEYSPSVQKTLYDIQVHSLSRVPEMEDMEISLPNIHYFNIDMSKMGLINKEEVLLPLDNPYGKITGTVKRKLSSRL

SEQ ID NO: 4 - protein, 304 aa, Artificial
  4
MAHYHNDYKKNDEVEFVRTGYGKDMVKVLHIQRDGKYHSIKEVATSVQLTLSSKKDYVYGDNSDIIPTDTIKNTVHVLAKFKGIKSIETFAMNICEHFLSSFNHVIRAQVYVEEVPWKRFEKNGVKHVHAFIHNPTGTHFCEVEQMRSGPPVIHSGIKDLKVLKTTQSGFEGFIKDQFTTLPEVKDRCFATKVYCKWRYHQGRDVDFEATWDTVRDIVLEKFAGPYDKGEYSPSVQKTLYDIQVHSLSRVPEMEDMEISLPNIHYFNIDMSKMGLINKEEVLLPLDNPYGRITGTAKRKLASKL

SEQ ID NO: 5 - protein, 304 aa, Artificial
  5
MAHYHNDYQKNDEVEFVRTGYGKDMVKVLHIQRDGKYHSIKEVATSVQLTLNSRREYLHGDNSDIIPTDTIKNTVQVLAKFKGIKSIETFAMNICEHFLSSFNHVIRVQVYVEEVPWKRFEKNGVKHVHAFIHTPTGTHFCEVEQLRSGPPVIHSGIKDLKVLKTTQSGFEGFLKDQFTTLPEVKDRCFATQVYCKWRYHQGRDVDFEATWEAVRGIVLKKFAGPYDKGEYSPSVQKTLYDIQVLSLSQLPEIEDMEISLPNIHYFNIDMSKMGLINKEEVLLPLDNPYGRITGTVKRKLTSRL

SEQ ID NO: 6 - protein, 304 aa, Artificial
  6
MAHYHNDYKKNDEVEFVRTGYGKDMVKVLHIQRDGKYHSIKEVATSVQLTLSSKKDYLHGDNSDIIPTDTIKNTVHALAKFKGIKSIEAFAVNICQHFLSSFNHVIRTQVYVEEIPWKRLEKNGVKHVHAFIHTPTGTHFCEVEQLRSGPPVIHSGIKDLKVLKTTQSGFEGFIKDQFTTLPEVKDRCFAAQVYCKWRYHQCRDVDFEATWDTIRDVVLEKFAGPYDKGEYSPSVQKTLYDIQVVSLSQVPEIDDMEISLPNIHYFNIDMSKMGLINKEEVLLPLDNPYGKITGTVKRKLSSRL

SEQ ID NO: 7 - protein, 304 aa, Artificial
  7
MADYHNNYKKNDELEFVRTGYGKDMVKVLHIQRDGKYHSIKEVATSVQLTLSSKKDYLHGDNSDIIPTDTIKNTVHVLAKFKGIKSIEAFGVNICEYFLSSFNHVIRAQVYVEEIPWKRLEKNGVKHVHAFIHTPTGTHFCEVEQLRSGPPVIHSGIKDLKVLKTTQSGFEGFIKDQFTTLPEVKDRCFATQVYCKWRYHQCRDVDFEATWGTIRDLVLEKFAGPYDKGEYSPSVQKTLYDIQVLSLSRVPEIEDMEISLPNIHYFNIDMSKMGLINKEEVLLPLDNPYGKITGTVKRKLSSRL